European Patent Specification EP 3 640 641 B1, published July 9, 2025. Title: A method for examining effect of cancer treatment  and a composition for  immune response induction. Applicant: Kawasaki Gakuen. The sequence listing filed with the application follows.

SEQUENCE LISTING (24 sequences)

SEQ ID NO: 1 - protein, 25 aa, Artificial Sequence
  A part of XAGE1
NQQLKVGILHLGSRQKKIRIQLRSQ

SEQ ID NO: 2 - protein, 25 aa, Artificial Sequence
  A part of XAGE1
ISQTPGINLDLGSGVKVKIIPKEEH

SEQ ID NO: 3 - protein, 81 aa, Homo sapiens
MESPKKKNQQLKVGILHLGSRQKKIRIQLRSQCATWKVICKSCISQTPGINLDLGSGVKVKIIPKEEHCKMPEAGEEQPQV

SEQ ID NO: 4 - protein, 180 aa, Homo sapiens
MQAEGRGTGGSTGDADGPGGPGIPDGPGGNAGGPGEAGATGGRGPRGAGAARASGPGGGAPRGPHGGAASGLNGCCRCGARGPESRLLEFYLAMPFATPMEAELARRSLAQDAPPLPVPGVLLKEFTVSGNILTIRLTAADHRQLQLSISSCLQQLSLLMWITQCFLPVFLAQPPSGQRR

SEQ ID NO: 5 - protein, 15 aa, Artificial Sequence
  1-15
MESPKKKNQQLKVGI

SEQ ID NO: 6 - protein, 15 aa, Artificial Sequence
  4-18
PKKKNQQLKVGILHL

SEQ ID NO: 7 - protein, 15 aa, Artificial Sequence
  7-21
KNQQLKVGILHLGSR

SEQ ID NO: 8 - protein, 15 aa, Artificial Sequence
  10-24
QLKVGILHLGSRQKK

SEQ ID NO: 9 - protein, 15 aa, Artificial Sequence
  13-27
VGILHLGSRQKKIRI

SEQ ID NO: 10 - protein, 15 aa, Artificial Sequence
  16-30
LHLGSRQKKIRIQLR

SEQ ID NO: 11 - protein, 15 aa, Artificial Sequence
  19-33
GSRQKKIRIQLRSQC

SEQ ID NO: 12 - protein, 15 aa, Artificial Sequence
  22-36
QKKIRIQLRSQCATW

SEQ ID NO: 13 - protein, 15 aa, Artificial Sequence
  25-39
IRIQLRSQCATWKVI

SEQ ID NO: 14 - protein, 15 aa, Artificial Sequence
  28-42
QLRSQCATWKVICKS

SEQ ID NO: 15 - protein, 15 aa, Artificial Sequence
  31-45
SQCATWKVICKSCIS

SEQ ID NO: 16 - protein, 15 aa, Artificial Sequence
  37-51
KVICKSCISQTPGIN

SEQ ID NO: 17 - protein, 15 aa, Artificial Sequence
  40-54
CKSCISQTPGINLDL

SEQ ID NO: 18 - protein, 15 aa, Artificial Sequence
  43-57
CISQTPGINLDLGSG

SEQ ID NO: 19 - protein, 15 aa, Artificial Sequence
  46-60
QTPGINLDLGSGVKV

SEQ ID NO: 20 - protein, 15 aa, Artificial Sequence
  49-63
GINLDLGSGVKVKII

SEQ ID NO: 21 - protein, 17 aa, Artificial Sequence
  52-68
LDLGSGVKVKIIPKEEH

SEQ ID NO: 22 - protein, 17 aa, Artificial Sequence
  55-71
GSGVKVKIIPKEEHCKM

SEQ ID NO: 23 - protein, 17 aa, Artificial Sequence
  58-74
VKVKIIPKEEHCKMPEA

SEQ ID NO: 24 - protein, 17 aa, Artificial Sequence
  61-77
KIIPKEEHCKMPEAGEE